European Patent Specification EP 3 590 966 B1, published March 5, 2025. Title: Anti-alpha2 integrin antibodies and their uses. Applicant: Sanofi. The sequence listing filed with the application follows.

SEQUENCE LISTING (57 sequences)

SEQ ID NO: 1 - protein, 10 aa, Artificial
  HCDR1 [CDR1 of heavy chain variable region]
GFSLTNYGIH

SEQ ID NO: 2 - protein, 16 aa, Artificial
  HCDR2  [CDR2 of heavy chain variable region]
VIWARGFTNYNSALMS

SEQ ID NO: 3 - protein, 11 aa, Artificial
  HCDR3  [CDR3 of heavy chain variable region]
ANDGVYYAMDY

SEQ ID NO: 4 - protein, 10 aa, Artificial
  LCDR1  [CDR1 of light chain variable region]
SAQSSVNYIH

SEQ ID NO: 5 - protein, 7 aa, Artificial
  LCDR2  [CDR2 of light chain variable region]
DTSKLAS

SEQ ID NO: 6 - protein, 9 aa, Artificial
  LCDR3  [CDR3 of light chain variable region]
QQWTTNPLT

SEQ ID NO: 7 - protein, 119 aa, Artificial
  humanized VH region
  VARIANT (30)..(30): Xaa at position 30 can be Thr or Ile
  VARIANT (31)..(31): Xaa at position 31 can be Asn or Ser
  VARIANT (37)..(37): Xaa at position 37 can be Val or Ile
  VARIANT (48)..(48): Xaa at position 48 can be Leu or Ile
  VARIANT (67)..(67): Xaa at position 67 can be Val or Leu
  VARIANT (71)..(71): Xaa at position 71 can be Lys or Val
  VARIANT (73)..(73): Xaa at position 73 can be Asn or Thr
  VARIANT (78)..(78): Xaa at position 78 can be Val or Phe
  VARIANT (94)..(94): Xaa at position 94 can be Phe or Tyr
QVQLQESGPGLVKPSETLSLTCTVSGFSLXXYGIHWXRQPPGKGLEWXGVIWARGFTNYNSALMSRXTISXDXSKNQXSLKLSSVTAADTAVYXCARANDGVYYAMDYWGQGTLVTVSS

SEQ ID NO: 8 - protein, 119 aa, Artificial
  humanizedVH2.0
QVQLQESGPGLVKPSETLSLTCTVSGFSLTNYGIHWVRQPPGKGLEWLGVIWARGFTNYNSALMSRVTISKDNSKNQVSLKLSSVTAADTAVYFCARANDGVYYAMDYWGQGTLVTVSS

SEQ ID NO: 9 - protein, 119 aa, Artificial
  humanizedVH3.0
QVQLQESGPGLVKPSETLSLTCTVSGFSLTNYGIHWVRQPPGKGLEWLGVIWARGFTNYNSALMSRVTISVDTSKNQFSLKLSSVTAADTAVYFCARANDGVYYAMDYWGQGTLVTVSS

SEQ ID NO: 10 - protein, 119 aa, Artificial
  humanizedVH4.0
QVQLQESGPGLVKPSETLSLTCTVSGFSLTNYGIHWIRQPPGKGLEWIGVIWARGFTNYNSALMSRLTISKDNSKNQVSLKLSSVTAADTAVYFCARANDGVYYAMDYWGQGTLVTVSS

SEQ ID NO: 11 - protein, 119 aa, Artificial
  humanizedVH5.0
QVQLQESGPGLVKPSETLSLTCTVSGFSLTNYGIHWVRQPPGKGLEWIGVIWARGFTNYNSALMSRLTISKDNSKNQVSLKLSSVTAADTAVYFCARANDGVYYAMDYWGQGTLVTVSS

SEQ ID NO: 12 - protein, 119 aa, Artificial
  humanizedVH6.0
QVQLQESGPGLVKPSETLSLTCTVSGFSLTNYGIHWVRQPPGKGLEWIGVIWARGFTNYNSALMSRVTISKDNSKNQVSLKLSSVTAADTAVYFCARANDGVYYAMDYWGQGTLVTVSS

SEQ ID NO: 13 - protein, 119 aa, Artificial
  humanizedVH7.0
QVQLQESGPGLVKPSETLSLTCTVSGFSLTNYGIHWVRQPPGKGLEWLGVIWARGFTNYNSALMSRLTISKDNSKNQVSLKLSSVTAADTAVYYCARANDGVYYAMDYWGQGTLVTVSS

SEQ ID NO: 14 - protein, 119 aa, Artificial
  humanizedVH9.0 Position 48 can be Leucine or Isoleucine
QVQLQESGPGLVKPSETLSLTCTVSGFSLTNYGIHWVRQPPGKGLEWIGVIWARGFTNYNSALMSRLTISVDNSKNQVSLKLSSVTAADTAVYFCARANDGVYYAMDYWGQGTLVTVSS

SEQ ID NO: 15 - protein, 119 aa, Artificial
  humanizedVH10.0
QVQLQESGPGLVKPSETLSLTCTVSGFSLTNYGIHWVRQPPGKGLEWLGVIWARGFTNYNSALMSRLTISKDTSKNQVSLKLSSVTAADTAVYFCARANDGVYYAMDYWGQGTLVTVSS

SEQ ID NO: 16 - protein, 119 aa, Artificial
  humanizedVH11.0  Position 48 can be Leucine or Isoleucine
QVQLQESGPGLVKPSETLSLTCTVSGFSLTNYGIHWVRQPPGKGLEWIGVIWARGFTNYNSALMSRLTISKDNSKNQFSLKLSSVTAADTAVYFCARANDGVYYAMDYWGQGTLVTVSS

SEQ ID NO: 17 - protein, 119 aa, Artificial
  humanizedVH12.0  Position 48 can be Leucine or Isoleucine
QVQLQESGPGLVKPSETLSLTCTVSGFSLTNYGIHWIRQPPGKGLEWLGVIWARGFTNYNSALMSRLTISKDNSKNQVSLKLSSVTAADTAVYYCARANDGVYYAMDYWGQGTLVTVSS

SEQ ID NO: 18 - protein, 119 aa, Artificial
  humanizedVH13.0
QVQLQESGPGLVKPSETLSLTCTVSGFSLTNYGIHWVRQPPGKGLEWIGVIWARGFTNYNSALMSRVTISKDNSKNQVSLKLSSVTAADTAVYYCARANDGVYYAMDYWGQGTLVTVSS

SEQ ID NO: 19 - protein, 119 aa, Artificial
  humanizedVH14.0 Position 48 can be Leucine or Isoleucine
QVQLQESGPGLVKPSETLSLTCTVSGFSLTNYGIHWIRQPPGKGLEWLGVIWARGFTNYNSALMSRVTISKDNSKNQVSLKLSSVTAADTAVYYCARANDGVYYAMDYWGQGTLVTVSS

SEQ ID NO: 20 - protein, 11 aa, Artificial
  FW4 4-59 [NCBI entry gi/33583]
WGQGTLVTVSS

SEQ ID NO: 21 - protein, 106 aa, Artificial
  humanized VL region
  VARIANT (1)..(1): Xaa at position 1 can be Gln or Asp
  VARIANT (2)..(2): Xaa at position 2 can be Phe or Val
  VARIANT (4)..(4): Xaa at position 4 can be Leu or Met
  VARIANT (45)..(45): Xaa at position 45 can be Lys or Leu
  VARIANT (46)..(46): Xaa at position 46 can be Trp or Leu
  VARIANT (48)..(48): Xaa at position 48 can be Tyr or Lys
  VARIANT (70)..(70): Xaa at position 70 can be Tyr or Phe
XXVXTQSPAFLSVTPGEKVTITCSAQSSVNYIHWYQQKPDQAPKXXIXDTSKLASGVPSRFSGSGSGTDXTFTISSLEAEDAATYYCQQWTTNPLTFGQGTKVEIK

SEQ ID NO: 22 - protein, 106 aa, Artificial
  humanizedVL2.0Q
QFVLTQSPAFLSVTPGEKVTITCSAQSSVNYIHWYQQKPDQAPKKLIYDTSKLASGVPSRFSGSGSGTDYTFTISSLEAEDAATYYCQQWTTNPLTFGQGTKVEIK

SEQ ID NO: 23 - protein, 106 aa, Artificial
  humanizedVL3.0Q
QFVLTQSPAFLSVTPGEKVTITCSAQSSVNYIHWYQQKPDQAPKLLIYDTSKLASGVPSRFSGSGSGTDYTFTISSLEAEDAATYYCQQWTTNPLTFGQGTKVEIK

SEQ ID NO: 24 - protein, 106 aa, Artificial
  humanizedVL4.0Q
DVVMTQSPAFLSVTPGEKVTITCSAQSSVNYIHWYQQKPDQAPKKWIYDTSKLASGVPSRFSGSGSGTDYTFTISSLEAEDAATYYCQQWTTNPLTFGQGTKVEIK

SEQ ID NO: 25 - protein, 106 aa, Artificial
  humanizedVL5.0Q
DFVLTQSPAFLSVTPGEKVTITCSAQSSVNYIHWYQQKPDQAPKKWIYDTSKLASGVPSRFSGSGSGTDYTFTISSLEAEDAATYYCQQWTTNPLTFGQGTKVEIK

SEQ ID NO: 26 - protein, 106 aa, Artificial
  humanizedVL6.0Q
QFVMTQSPAFLSVTPGEKVTITCSAQSSVNYIHWYQQKPDQAPKKWIYDTSKLASGVPSRFSGSGSGTDYTFTISSLEAEDAATYYCQQWTTNPLTFGQGTKVEIK

SEQ ID NO: 27 - protein, 106 aa, Artificial
  humanizedVL7.0Q
DFVMTQSPAFLSVTPGEKVTITCSAQSSVNYIHWYQQKPDQAPKKWIYDTSKLASGVPSRFSGSGSGTDYTFTISSLEAEDAATYYCQQWTTNPLTFGQGTKVEIK

SEQ ID NO: 28 - protein, 106 aa, Artificial
  humanizedVL8.0Q
QFVLTQSPAFLSVTPGEKVTITCSAQSSVNYIHWYQQKPDQAPKKWIYDTSKLASGVPSRFSGSGSGTDFTFTISSLEAEDAATYYCQQWTTNPLTFGQGTKVEIK

SEQ ID NO: 29 - protein, 106 aa, Artificial
  humanizedVL9.0Q
QFVLTQSPAFLSVTPGEKVTITCSAQSSVNYIHWYQQKPDQAPKKWIKDTSKLASGVPSRFSGSGSGTDYTFTISSLEAEDAATYYCQQWTTNPLTFGQGTKVEIK

SEQ ID NO: 30 - protein, 106 aa, Artificial
  humanizedVL10.0Q
DFVMTQSPAFLSVTPGEKVTITCSAQSSVNYIHWYQQKPDQAPKKLIYDTSKLASGVPSRFSGSGSGTDYTFTISSLEAEDAATYYCQQWTTNPLTFGQGTKVEIK

SEQ ID NO: 31 - protein, 106 aa, Artificial
  humanizedVL11.0Q
DFVMTQSPAFLSVTPGEKVTITCSAQSSVNYIHWYQQKPDQAPKKWIYDTSKLASGVPSRFSGSGSGTDFTFTISSLEAEDAATYYCQQWTTNPLTFGQGTKVEIK

SEQ ID NO: 32 - protein, 106 aa, Artificial
  humanizedVL1.0Q
QFVLTQSPAFLSVTPGEKVTITCSAQSSVNYIHWYQQKPDQAPKKWIYDTSKLASGVPSRFSGSGSGTDYTFTISSLEAEDAATYYCQQWTTNPLTFGQGTKVEIK

SEQ ID NO: 33 - protein, 106 aa, Artificial
  humanizedVL12.0Q
DFVMTQSPAFLSVTPGEKVTITCSAQSSVNYIHWYQQKPDQAPKKLIYDTSKLASGVPSRFSGSGSGTDFTFTISSLEAEDAATYYCQQWTTNPLTFGQGTKVEIK

SEQ ID NO: 34 - protein, 10 aa, Artificial
  FW 4 of mature kappa light chain
FGQGTKVEIK

SEQ ID NO: 35 - protein, 330 aa, Artificial
  variant human IgG 1133 heavy chain constant region
ASTKGPSVFPLAPSSKSTSGGTAALGCLVKDYFPEPVTVSWNSGALTSGVHTFPAVLQSSGLYSLSSVVTVPSSSLGTQTYICNVNHKPSNTKVDKKVEPKSCDKTHTCPPCPAPELLGGPSVFLFPPKPKDTLMISRTPEVTCVVVDVSHEDPEVQFKWYVDGVEVHNAKTKPREEQYNSTFRVVSVLTVLHQDWLNGKEYKCKVSNKALPAPIEKTISKTKGQPREPQVYTLPPSREEMTKNQVSLTCLVKGFYPSDIAVEWESSGQPENNYNTTPPMLDSDGSFFLYSKLTVDKSRWQQGNIFSCSVMHEALHNRFTQKSLSLSPGK

SEQ ID NO: 36 - protein, 330 aa, Artificial
  variant human IgG 3133 heavy chain constant region
ASTKGPSVFPLAPCSRSTSGGTAALGCLVKDYFPEPVTVSWNSGALTSGVHTFPAVLQSSGLYSLSSVVTVPSSSLGTQTYTCNVNHKPSNTKVDKRVEPKSCDKTHTCPPCPAPELLGGPSVFLFPPKPKDTLMISRTPEVTCVVVDVSHEDPEVQFKWYVDGVEVHNAKTKPREEQYNSTFRVVSVLTVLHQDWLNGKEYKCKVSNKALPAPIEKTISKTKGQPREPQVYTLPPSREEMTKNQVSLTCLVKGFYPSDIAVEWESSGQPENNYNTTPPMLDSDGSFFLYSKLTVDKSRWQQGNIFSCSVMHEALHNRFTQKSLSLSPGK

SEQ ID NO: 37 - protein, 330 aa, Artificial
  variant human IgG1 heavy chain constant region  E269D
ASTKGPSVFPLAPSSKSTSGGTAALGCLVKDYFPEPVTVSWNSGALTSGVHTFPAVLQSSGLYSLSSVVTVPSSSLGTQTYICNVNHKPSNTKVDKKVEPKSCDKTHTCPPCPAPELLGGPSVFLFPPKPKDTLMISRTPEVTCVVVDVSHDDPEVKFNWYVDGVEVHNAKTKPREEQYNSTYRVVSVLTVLHQDWLNGKEYKCKVSNKALPAPIEKTISKAKGQPREPQVYTLPPSRDELTKNQVSLTCLVKGFYPSDIAVEWESNGQPENNYKTTPPVLDSDGSFFLYSKLTVDKSRWQQGNVFSCSVMHEALHNHYTQKSLSLSPGK

SEQ ID NO: 38 - protein, 330 aa, Artificial
  variant human IgG1 heavy chain constant region  S298A
ASTKGPSVFPLAPSSKSTSGGTAALGCLVKDYFPEPVTVSWNSGALTSGVHTFPAVLQSSGLYSLSSVVTVPSSSLGTQTYICNVNHKPSNTKVDKKVEPKSCDKTHTCPPCPAPELLGGPSVFLFPPKPKDTLMISRTPEVTCVVVDVSHEDPEVKFNWYVDGVEVHNAKTKPREEQYNATYRVVSVLTVLHQDWLNGKEYKCKVSNKALPAPIEKTISKAKGQPREPQVYTLPPSRDELTKNQVSLTCLVKGFYPSDIAVEWESNGQPENNYKTTPPVLDSDGSFFLYSKLTVDKSRWQQGNVFSCSVMHEALHNHYTQKSLSLSPGK

SEQ ID NO: 39 - protein, 330 aa, Artificial
  variant human IgG1 heavy chain constant region  S324N
ASTKGPSVFPLAPSSKSTSGGTAALGCLVKDYFPEPVTVSWNSGALTSGVHTFPAVLQSSGLYSLSSVVTVPSSSLGTQTYICNVNHKPSNTKVDKKVEPKSCDKTHTCPPCPAPELLGGPSVFLFPPKPKDTLMISRTPEVTCVVVDVSHEDPEVKFNWYVDGVEVHNAKTKPREEQYNSTYRVVSVLTVLHQDWLNGKEYKCKVNNKALPAPIEKTISKAKGQPREPQVYTLPPSRDELTKNQVSLTCLVKGFYPSDIAVEWESNGQPENNYKTTPPVLDSDGSFFLYSKLTVDKSRWQQGNVFSCSVMHEALHNHYTQKSLSLSPGK

SEQ ID NO: 40 - protein, 330 aa, Artificial
  variant human IgG1 heavy chain constant region  E269D/S298A
ASTKGPSVFPLAPSSKSTSGGTAALGCLVKDYFPEPVTVSWNSGALTSGVHTFPAVLQSSGLYSLSSVVTVPSSSLGTQTYICNVNHKPSNTKVDKKVEPKSCDKTHTCPPCPAPELLGGPSVFLFPPKPKDTLMISRTPEVTCVVVDVSHDDPEVKFNWYVDGVEVHNAKTKPREEQYNATYRVVSVLTVLHQDWLNGKEYKCKVSNKALPAPIEKTISKAKGQPREPQVYTLPPSRDELTKNQVSLTCLVKGFYPSDIAVEWESNGQPENNYKTTPPVLDSDGSFFLYSKLTVDKSRWQQGNVFSCSVMHEALHNHYTQKSLSLSPGK

SEQ ID NO: 41 - protein, 330 aa, Artificial
  variant human IgG1 heavy chain constant region  E269D/S324N
ASTKGPSVFPLAPSSKSTSGGTAALGCLVKDYFPEPVTVSWNSGALTSGVHTFPAVLQSSGLYSLSSVVTVPSSSLGTQTYICNVNHKPSNTKVDKKVEPKSCDKTHTCPPCPAPELLGGPSVFLFPPKPKDTLMISRTPEVTCVVVDVSHDDPEVKFNWYVDGVEVHNAKTKPREEQYNSTYRVVSVLTVLHQDWLNGKEYKCKVNNKALPAPIEKTISKAKGQPREPQVYTLPPSRDELTKNQVSLTCLVKGFYPSDIAVEWESNGQPENNYKTTPPVLDSDGSFFLYSKLTVDKSRWQQGNVFSCSVMHEALHNHYTQKSLSLSPGK

SEQ ID NO: 42 - protein, 330 aa, Artificial
  variant human IgG1 heavy chain constant region  S298A/S324N
ASTKGPSVFPLAPSSKSTSGGTAALGCLVKDYFPEPVTVSWNSGALTSGVHTFPAVLQSSGLYSLSSVVTVPSSSLGTQTYICNVNHKPSNTKVDKKVEPKSCDKTHTCPPCPAPELLGGPSVFLFPPKPKDTLMISRTPEVTCVVVDVSHEDPEVKFNWYVDGVEVHNAKTKPREEQYNATYRVVSVLTVLHQDWLNGKEYKCKVNNKALPAPIEKTISKAKGQPREPQVYTLPPSRDELTKNQVSLTCLVKGFYPSDIAVEWESNGQPENNYKTTPPVLDSDGSFFLYSKLTVDKSRWQQGNVFSCSVMHEALHNHYTQKSLSLSPGK

SEQ ID NO: 43 - protein, 330 aa, Artificial
  variant human IgG1 heavy chain constant region  E269D/S298A/S324N
ASTKGPSVFPLAPSSKSTSGGTAALGCLVKDYFPEPVTVSWNSGALTSGVHTFPAVLQSSGLYSLSSVVTVPSSSLGTQTYICNVNHKPSNTKVDKKVEPKSCDKTHTCPPCPAPELLGGPSVFLFPPKPKDTLMISRTPEVTCVVVDVSHDDPEVKFNWYVDGVEVHNAKTKPREEQYNATYRVVSVLTVLHQDWLNGKEYKCKVNNKALPAPIEKTISKAKGQPREPQVYTLPPSRDELTKNQVSLTCLVKGFYPSDIAVEWESNGQPENNYKTTPPVLDSDGSFFLYSKLTVDKSRWQQGNVFSCSVMHEALHNHYTQKSLSLSPGK

SEQ ID NO: 44 - protein, 449 aa, Artificial
  heavy chain anti-VLA2 IgG1
QVQLQESGPGLVKPSETLSLTCTVSGFSLTNYGIHWIRQPPGKGLEWLGVIWARGFTNYNSALMSRLTISKDNSKNQVSLKLSSVTAADTAVYYCARANDGVYYAMDYWGQGTLVTVSSASTKGPSVFPLAPSSKSTSGGTAALGCLVKDYFPEPVTVSWNSGALTSGVHTFPAVLQSSGLYSLSSVVTVPSSSLGTQTYICNVNHKPSNTKVDKKVEPKSCDKTHTCPPCPAPELLGGPSVFLFPPKPKDTLMISRTPEVTCVVVDVSHEDPEVKFNWYVDGVEVHNAKTKPREEQYNSTYRVVSVLTVLHQDWLNGKEYKCKVSNKALPAPIEKTISKAKGQPREPQVYTLPPSRDELTKNQVSLTCLVKGFYPSDIAVEWESNGQPENNYKTTPPVLDSDGSFFLYSKLTVDKSRWQQGNVFSCSVMHEALHNHYTQKSLSLSPGK

SEQ ID NO: 45 - protein, 445 aa, Artificial
  heavy chain anti-VLA2 IgG2
QVQLQESGPGLVKPSETLSLTCTVSGFSLTNYGIHWIRQPPGKGLEWLGVIWARGFTNYNSALMSRLTISKDNSKNQVSLKLSSVTAADTAVYYCARANDGVYYAMDYWGQGTLVTVSSASTKGPSVFPLAPCSRSTSESTAALGCLVKDYFPEPVTVSWNSGALTSGVHTFPAVLQSSGLYSLSSVVTVPSSNFGTQTYTCNVDHKPSNTKVDKTVERKCCVECPPCPAPPVAGPSVFLFPPKPKDTLMISRTPEVTCVVVDVSHEDPEVQFNWYVDGVEVHNAKTKPREEQFNSTFRVVSVLTVVHQDWLNGKEYKCKVSNKGLPAPIEKTISKTKGQPREPQVYTLPPSREEMTKNQVSLTCLVKGFYPSDIAVEWESNGQPENNYKTTPPMLDSDGSFFLYSKLTVDKSRWQQGNVFSCSVMHEALHNHYTQKSLSLSPGK

SEQ ID NO: 46 - protein, 496 aa, Artificial
  heavy chain anti-VLA2 IgG3
QVQLQESGPGLVKPSETLSLTCTVSGFSLTNYGIHWIRQPPGKGLEWLGVIWARGFTNYNSALMSRLTISKDNSKNQVSLKLSSVTAADTAVYYCARANDGVYYAMDYWGQGTLVTVSSASTKGPSVFPLAPCSRSTSGGTAALGCLVKDYFPEPVTVSWNSGALTSGVHTFPAVLQSSGLYSLSSVVTVPSSSLGTQTYTCNVNHKPSNTKVDKRVELKTPLGDTTHTCPRCPEPKSCDTPPPCPRCPEPKSCDTPPPCPRCPEPKSCDTPPPCPRCPAPELLGGPSVFLFPPKPKDTLMISRTPEVTCVVVDVSHEDPEVQFKWYVDGVEVHNAKTKPREEQYNSTFRVVSVLTVLHQDWLNGKEYKCKVSNKALPAPIEKTISKTKGQPREPQVYTLPPSREEMTKNQVSLTCLVKGFYPSDIAVEWESSGQPENNYNTTPPMLDSDGSFFLYSKLTVDKSRWQQGNIFSCSVMHEALHNRFTQKSLSLSPGK

SEQ ID NO: 47 - protein, 449 aa, Artificial
  heavy chain anti-VLA2 IgG (1133)
QVQLQESGPGLVKPSETLSLTCTVSGFSLTNYGIHWIRQPPGKGLEWLGVIWARGFTNYNSALMSRLTISKDNSKNQVSLKLSSVTAADTAVYYCARANDGVYYAMDYWGQGTLVTVSSASTKGPSVFPLAPSSKSTSGGTAALGCLVKDYFPEPVTVSWNSGALTSGVHTFPAVLQSSGLYSLSSVVTVPSSSLGTQTYICNVNHKPSNTKVDKKVEPKSCDKTHTCPPCPAPELLGGPSVFLFPPKPKDTLMISRTPEVTCVVVDVSHEDPEVQFKWYVDGVEVHNAKTKPREEQYNSTFRVVSVLTVLHQDWLNGKEYKCKVSNKALPAPIEKTISKTKGQPREPQVYTLPPSREEMTKNQVSLTCLVKGFYPSDIAVEWESSGQPENNYNTTPPMLDSDGSFFLYSKLTVDKSRWQQGNIFSCSVMHEALHNRFTQKSLSLSPGK

SEQ ID NO: 48 - protein, 449 aa, Artificial
  heavy chain anti-VLA2 IgG (3133)
QVQLQESGPGLVKPSETLSLTCTVSGFSLTNYGIHWIRQPPGKGLEWLGVIWARGFTNYNSALMSRLTISKDNSKNQVSLKLSSVTAADTAVYYCARANDGVYYAMDYWGQGTLVTVSSASTKGPSVFPLAPCSRSTSGGTAALGCLVKDYFPEPVTVSWNSGALTSGVHTFPAVLQSSGLYSLSSVVTVPSSSLGTQTYTCNVNHKPSNTKVDKRVEPKSCDKTHTCPPCPAPELLGGPSVFLFPPKPKDTLMISRTPEVTCVVVDVSHEDPEVQFKWYVDGVEVHNAKTKPREEQYNSTFRVVSVLTVLHQDWLNGKEYKCKVSNKALPAPIEKTISKTKGQPREPQVYTLPPSREEMTKNQVSLTCLVKGFYPSDIAVEWESSGQPENNYNTTPPMLDSDGSFFLYSKLTVDKSRWQQGNIFSCSVMHEALHNRFTQKSLSLSPGK

SEQ ID NO: 49 - protein, 449 aa, Artificial
  heavy chain anti-VLA2 IgG1 S324N
QVQLQESGPGLVKPSETLSLTCTVSGFSLTNYGIHWIRQPPGKGLEWLGVIWARGFTNYNSALMSRLTISKDNSKNQVSLKLSSVTAADTAVYYCARANDGVYYAMDYWGQGTLVTVSSASTKGPSVFPLAPSSKSTSGGTAALGCLVKDYFPEPVTVSWNSGALTSGVHTFPAVLQSSGLYSLSSVVTVPSSSLGTQTYICNVNHKPSNTKVDKKVEPKSCDKTHTCPPCPAPELLGGPSVFLFPPKPKDTLMISRTPEVTCVVVDVSHEDPEVKFNWYVDGVEVHNAKTKPREEQYNSTYRVVSVLTVLHQDWLNGKEYKCKVNNKALPAPIEKTISKAKGQPREPQVYTLPPSRDELTKNQVSLTCLVKGFYPSDIAVEWESNGQPENNYKTTPPVLDSDGSFFLYSKLTVDKSRWQQGNVFSCSVMHEALHNHYTQKSLSLSPGK

SEQ ID NO: 50 - protein, 449 aa, Artificial
  heavy chain anti-VLA2 IgG1 E269D
QVQLQESGPGLVKPSETLSLTCTVSGFSLTNYGIHWIRQPPGKGLEWLGVIWARGFTNYNSALMSRLTISKDNSKNQVSLKLSSVTAADTAVYYCARANDGVYYAMDYWGQGTLVTVSSASTKGPSVFPLAPSSKSTSGGTAALGCLVKDYFPEPVTVSWNSGALTSGVHTFPAVLQSSGLYSLSSVVTVPSSSLGTQTYICNVNHKPSNTKVDKKVEPKSCDKTHTCPPCPAPELLGGPSVFLFPPKPKDTLMISRTPEVTCVVVDVSHDDPEVKFNWYVDGVEVHNAKTKPREEQYNSTYRVVSVLTVLHQDWLNGKEYKCKVSNKALPAPIEKTISKAKGQPREPQVYTLPPSRDELTKNQVSLTCLVKGFYPSDIAVEWESNGQPENNYKTTPPVLDSDGSFFLYSKLTVDKSRWQQGNVFSCSVMHEALHNHYTQKSLSLSPGK

SEQ ID NO: 51 - protein, 449 aa, Artificial
  heavy chain anti-VLA2 IgG1 S298A
QVQLQESGPGLVKPSETLSLTCTVSGFSLTNYGIHWIRQPPGKGLEWLGVIWARGFTNYNSALMSRLTISKDNSKNQVSLKLSSVTAADTAVYYCARANDGVYYAMDYWGQGTLVTVSSASTKGPSVFPLAPSSKSTSGGTAALGCLVKDYFPEPVTVSWNSGALTSGVHTFPAVLQSSGLYSLSSVVTVPSSSLGTQTYICNVNHKPSNTKVDKKVEPKSCDKTHTCPPCPAPELLGGPSVFLFPPKPKDTLMISRTPEVTCVVVDVSHEDPEVKFNWYVDGVEVHNAKTKPREEQYNATYRVVSVLTVLHQDWLNGKEYKCKVSNKALPAPIEKTISKAKGQPREPQVYTLPPSRDELTKNQVSLTCLVKGFYPSDIAVEWESNGQPENNYKTTPPVLDSDGSFFLYSKLTVDKSRWQQGNVFSCSVMHEALHNHYTQKSLSLSPGK

SEQ ID NO: 52 - protein, 449 aa, Artificial
  heavy chain anti-VLA2 IgG1 E269D/S298A
QVQLQESGPGLVKPSETLSLTCTVSGFSLTNYGIHWIRQPPGKGLEWLGVIWARGFTNYNSALMSRLTISKDNSKNQVSLKLSSVTAADTAVYYCARANDGVYYAMDYWGQGTLVTVSSASTKGPSVFPLAPSSKSTSGGTAALGCLVKDYFPEPVTVSWNSGALTSGVHTFPAVLQSSGLYSLSSVVTVPSSSLGTQTYICNVNHKPSNTKVDKKVEPKSCDKTHTCPPCPAPELLGGPSVFLFPPKPKDTLMISRTPEVTCVVVDVSHDDPEVKFNWYVDGVEVHNAKTKPREEQYNATYRVVSVLTVLHQDWLNGKEYKCKVSNKALPAPIEKTISKAKGQPREPQVYTLPPSRDELTKNQVSLTCLVKGFYPSDIAVEWESNGQPENNYKTTPPVLDSDGSFFLYSKLTVDKSRWQQGNVFSCSVMHEALHNHYTQKSLSLSPGK

SEQ ID NO: 53 - protein, 449 aa, Artificial
  heavy chain anti-VLA2 IgG1 E269D/S324N
QVQLQESGPGLVKPSETLSLTCTVSGFSLTNYGIHWIRQPPGKGLEWLGVIWARGFTNYNSALMSRLTISKDNSKNQVSLKLSSVTAADTAVYYCARANDGVYYAMDYWGQGTLVTVSSASTKGPSVFPLAPSSKSTSGGTAALGCLVKDYFPEPVTVSWNSGALTSGVHTFPAVLQSSGLYSLSSVVTVPSSSLGTQTYICNVNHKPSNTKVDKKVEPKSCDKTHTCPPCPAPELLGGPSVFLFPPKPKDTLMISRTPEVTCVVVDVSHDDPEVKFNWYVDGVEVHNAKTKPREEQYNSTYRVVSVLTVLHQDWLNGKEYKCKVNNKALPAPIEKTISKAKGQPREPQVYTLPPSRDELTKNQVSLTCLVKGFYPSDIAVEWESNGQPENNYKTTPPVLDSDGSFFLYSKLTVDKSRWQQGNVFSCSVMHEALHNHYTQKSLSLSPGK

SEQ ID NO: 54 - protein, 449 aa, Artificial
  heavy chain anti-VLA2 IgG1 S298A/S324N
QVQLQESGPGLVKPSETLSLTCTVSGFSLTNYGIHWIRQPPGKGLEWLGVIWARGFTNYNSALMSRLTISKDNSKNQVSLKLSSVTAADTAVYYCARANDGVYYAMDYWGQGTLVTVSSASTKGPSVFPLAPSSKSTSGGTAALGCLVKDYFPEPVTVSWNSGALTSGVHTFPAVLQSSGLYSLSSVVTVPSSSLGTQTYICNVNHKPSNTKVDKKVEPKSCDKTHTCPPCPAPELLGGPSVFLFPPKPKDTLMISRTPEVTCVVVDVSHEDPEVKFNWYVDGVEVHNAKTKPREEQYNATYRVVSVLTVLHQDWLNGKEYKCKVNNKALPAPIEKTISKAKGQPREPQVYTLPPSRDELTKNQVSLTCLVKGFYPSDIAVEWESNGQPENNYKTTPPVLDSDGSFFLYSKLTVDKSRWQQGNVFSCSVMHEALHNHYTQKSLSLSPGK

SEQ ID NO: 55 - protein, 449 aa, Artificial
  heavy chain anti-VLA2 IgG1 E269D/S298A/S324N
QVQLQESGPGLVKPSETLSLTCTVSGFSLTNYGIHWIRQPPGKGLEWLGVIWARGFTNYNSALMSRLTISKDNSKNQVSLKLSSVTAADTAVYYCARANDGVYYAMDYWGQGTLVTVSSASTKGPSVFPLAPSSKSTSGGTAALGCLVKDYFPEPVTVSWNSGALTSGVHTFPAVLQSSGLYSLSSVVTVPSSSLGTQTYICNVNHKPSNTKVDKKVEPKSCDKTHTCPPCPAPELLGGPSVFLFPPKPKDTLMISRTPEVTCVVVDVSHDDPEVKFNWYVDGVEVHNAKTKPREEQYNATYRVVSVLTVLHQDWLNGKEYKCKVNNKALPAPIEKTISKAKGQPREPQVYTLPPSRDELTKNQVSLTCLVKGFYPSDIAVEWESNGQPENNYKTTPPVLDSDGSFFLYSKLTVDKSRWQQGNVFSCSVMHEALHNHYTQKSLSLSPGK

SEQ ID NO: 56 - protein, 213 aa, Artificial
  light chain anti-VLA2 IgG4
DFVMTQSPAFLSVTPGEKVTITCSAQSSVNYIHWYQQKPDQAPKKLIYDTSKLASGVPSRFSGSGSGTDYTFTISSLEAEDAATYYCQQWTTNPLTFGQGTKVEIKRTVAAPSVFIFPPSDEQLKSGTASVVCLLNNFYPREAKVQWKVDNALQSGNSQESVTEQDSKDSTYSLSSTLTLSKADYEKHKVYACEVTHQGLSSPVTKSFNRGEC

SEQ ID NO: 57 - protein, 446 aa, Artificial
  heavy chain anti-VLA2 IgG4
QVQLQESGPGLVKPSETLSLTCTVSGFSLTNYGIHWIRQPPGKGLEWLGVIWARGFTNYNSALMSRLTISKDNSKNQVSLKLSSVTAADTAVYYCARANDGVYYAMDYWGQGTLVTVSSASTKGPSVFPLAPCSRSTSESTAALGCLVKDYFPEPVTVSWNSGALTSGVHTFPAVLQSSGLYSLSSVVTVPSSSLGTKTYTCNVDHKPSNTKVDKRVESKYGPPCPSCPAPEFLGGPSVFLFPPKPKDTLMISRTPEVTCVVVDVSQEDPEVQFNWYVDGVEVHNAKTKPREEQFNSTYRVVSVLTVLHQDWLNGKEYKCKVSNKGLPSSIEKTISKAKGQPREPQVYTLPPSQEEMTKNQVSLTCLVKGFYPSDIAVEWESNGQPENNYKTTPPVLDSDGSFFLYSRLTVDKSRWQEGNVFSCSVMHEALHNHYTQKSLSLSLGK